European Patent Application EP 4 332 220 A1, published March 6, 2024. Title: Method for amplifying target gene with specific GC content. Applicant: Denka Company Limited, Toho University. The sequence listing filed with the application follows.

SEQUENCE LISTING (24 sequences)

SEQ ID NO: 1 - DNA, 507 bp, Pseudomonas aeruginosa strain E6130952
ttacttcttcagctcgacgcgacggttctgagcccaggactgctcgtcgtggccggtagcgaccggacgctctttaccataggaaaccagttccagctgggccggcgaaacgccctgcagcaccaggtagcgctgaacggccttggcacgacgctcgcccagagccatgttgtactcgcgggtgccgcgttcgtcggtgtggccttccagcactacgcgctgaccgctgcctttcaggtctttcgcgtgtacgtccagagcgcgcatggcttccggcttcaggtcggagctgtcgtactcgaagtagaaggtggtgatcgcacgcagagcggcttcgtcgctcaggctgccgtcaacggcaccgctgttggcgccatagcctgcgttcgggtcgacgccgccattggcaccttcaccggaagcatcgccgcccttggaggagcaacccacagccacagccatggccagagccagcgcagcaaatttgccgaatttcagcatttccat

SEQ ID NO: 2 - DNA, 507 bp, Pseudomonas aeruginosa strain NCTC10332; identical to SEQ ID NO: 1

SEQ ID NO: 3 - DNA, 507 bp, Pseudomonas aeruginosa strain PAO1
ttacttcttcagctcgacgcgacggttctgagcccaggactgctcgtcgtggccggtagcgaccggacgctctttaccataggaaaccagttccagctgggccggcgaaacaccctgcagcaccaggtagcgctgaacggccttggcacgacgctcgcccagagccatattgtactcgcgggtgccgcgttcgtcggtgtggccttccagcactacgcgctgaccgctgcctttcaggtctttcgcgtgtacgtccagagcgcgcatggcttccggcttcaggtcggagctgtcgtactcgaagtagaaggtggtgatcgcacgcagagcggcttcgtcgctcaggctgccgtcaacggcaccgctgttggcgccatagcctgcgttcgggtcgacgccgccattggcaccttcaccggaagcatcgccgcccttggaggagcaacccacagccacagccatggccagagccagcgcagcaaatttgccgaatttcagcatttccat

SEQ ID NO: 4 - DNA, 18 bp, Artificial Sequence
  Forward primer for Pseudomonas aeruginosa
ggtaaagagcgtccggtc

SEQ ID NO: 5 - DNA, 19 bp, Artificial Sequence
  Reverse primer for Pseudomonas aeruginosa
ttacttcttcagctcgacg

SEQ ID NO: 6 - DNA, 25 bp, Artificial Sequence
  Probe for Pseudomonas aeruginosa
ttttttttttggtaaagagcgtccg

SEQ ID NO: 7 - DNA, 20 bp, Artificial Sequence
  Forward primer for Staphylococcus epidermidis
tacatyccaactccagaacg

SEQ ID NO: 8 - DNA, 20 bp, Artificial Sequence
  Reverse primer for Staphylococcus epidermidis
actttgatttgaccacgttc

SEQ ID NO: 9 - DNA, 25 bp, Artificial Sequence
  Probe for Staphylococcus epidermidis
tttttttttaaccattcatgatgcc

SEQ ID NO: 10 - DNA, 20 bp, Artificial Sequence
  Forward primer for Proteus mirabilis
caactcactayggtcgtgtg

SEQ ID NO: 11 - DNA, 22 bp, Artificial Sequence
  Reverse primer for Proteus mirabilis
catctgttacagcgttgttttc

SEQ ID NO: 12 - DNA, 25 bp, Artificial Sequence
  Probe for Proteus mirabilis
ttttttttttagaaacgccttaccg

SEQ ID NO: 13 - DNA, 23 bp, Artificial Sequence
  Forward primer for Acinetobacter baumannii
tgatctgacgaagacacattaac

SEQ ID NO: 14 - DNA, 22 bp, Artificial Sequence
  Reverse primer for Acinetobacter baumannii
atttcagtttagagcactgtgc

SEQ ID NO: 15 - DNA, 25 bp, Artificial Sequence
  Probe for Acinetobacter baumannii
ttttttgaatttagattgaagctgt

SEQ ID NO: 16 - DNA, 78 bp, Pseudomonas aeruginosa
ttacttcttcagctcgacgcgacggttctgagcccaggactgctcgtcgtggccggtagcgaccggacgctctttacc

SEQ ID NO: 17 - DNA, 122 bp, Staphylococcus epidermidis
tacattccaactccagaacgtgattctgacaaaccattcatgatgccagttgaggacgtattctcaatcactggtcgtggtactgttgctacaggccgtgttgaacgtggtcaaatcaaagt

SEQ ID NO: 18 - DNA, 150 bp, Proteus mirabilis
caactcactatggtcgtgtgtgtccaatcgaaacacctgaaggtccaaatatcggtctgattaactcattatctgtttatgcacagactaacgagtacggattcttagaaacgccttaccgtgttgtagaaaacaacgctgtaacagatg

SEQ ID NO: 19 - DNA, 198 bp, Acinetobacter baumannii
tgatctgacgaagacacattaactcattaacagattggcaaaattgagtctgaaataaattgttcactcaagagtttaggttaagcaattaatctagatgaattgagaactagcaaattaactgaatcaagcgttttggtatgtgaatttagattgaagctgtacggtgcttaagtgcacagtgctctaaactgaaat

SEQ ID NO: 20 - DNA, 25 bp, Artificial Sequence
  Primer for Enterococcus casseliflavus
ttcaattaaatttggtaattccaat

SEQ ID NO: 21 - DNA, 24 bp, Artificial Sequence
  Primer for Enterococcus casseliflavus
tcaatcaaattcggtaattcyaat

SEQ ID NO: 22 - DNA, 23 bp, Artificial Sequence
  Primer for Enterococcus casseliflavus
cgatcaaattyggtaattccaac

SEQ ID NO: 23 - DNA, 18 bp, Artificial Sequence
  Primer for Enterococcus casseliflavus
arcttggctggacacgta

SEQ ID NO: 24 - DNA, 15 bp, Artificial Sequence
  Probe for Enterococcus casseliflavus
gcttctacgttctcg